European Patent Specification EP 3 741 845 B1, published June 18, 2025. Title: RECOMBINANT VACCINIA VIRUS AND PHARMACECUTICAL COMPOSITON COMPRISING SAME. Applicant: KOLON LIFE SCIENCE, INC. The sequence listing filed with the application follows.

SEQUENCE LISTING (146 sequences)

SEQ ID NO: 1 - DNA, 36 bp, Artificial Sequence
  VGF-L forward primer (IHD-W)
cgaaagcttgtaagatgtttagaaaatggatatttc

SEQ ID NO: 2 - DNA, 52 bp, Artificial Sequence
  VGF-L reverse primer (IHD-W)
ctgggatcctaggctagcgtgtaaataatataaaaataacaatacaatattg

SEQ ID NO: 3 - DNA, 58 bp, Artificial Sequence
  VGF-R forward primer (IHD-W)
ctggaattcgatttaattaatttttataaattttttttatgagtatttttacaaaaaa

SEQ ID NO: 4 - DNA, 38 bp, Artificial Sequence
  VGF-R reverse primer (IHD-W)
tagggatcccatcgatagtacaataacttttatgaaat

SEQ ID NO: 5 - DNA, 30 bp, Artificial Sequence
  TK-L forward primer (IHD-W)
gatctgcagccctcttcaagaacccattag

SEQ ID NO: 6 - DNA, 51 bp, Artificial Sequence
  TK-L reverse primer (IHD-W)
tagggatcctaggcggccgcatgacaataaagaattaattattgttcactt

SEQ ID NO: 7 - DNA, 46 bp, Artificial Sequence
  TK-R forward primer (IHD-W)
catgaattctattatattttttatctaaaaaactaaaaataaacat

SEQ ID NO: 8 - DNA, 36 bp, Artificial Sequence
  TK-R reverse primer(IHD-W)
agatctatcgctttagtagtaggaaatgttttattg

SEQ ID NO: 9 - DNA, 35 bp, Artificial Sequence
  K3L-L forward primer (IHD-W)
tcggtcgaccatatgtttaaacgacgcattatctg

SEQ ID NO: 10 - DNA, 43 bp, Artificial Sequence
  K3L-L reverse primer (IHD-W)
tcgaagctttttttataccgaacataaaaataaggttaattat

SEQ ID NO: 11 - DNA, 34 bp, Artificial Sequence
  K3L-R forward primer (IHD-W)
cgcagataaaaatcacttgttaacgggctcgtaa

SEQ ID NO: 12 - DNA, 34 bp, Artificial Sequence
  K3L-R reverse primer (IHD-W)
aagcgctaacatggattaggaagcgctaacatgg

SEQ ID NO: 13 - DNA, 31 bp, Artificial Sequence
  p7.5-DsRed  forward primer (IHD-W)
aggaagctttccaaacccacccgctttttat

SEQ ID NO: 14 - DNA, 28 bp, Artificial Sequence
  p7.5-DsRed reverse primer (IHD-W)
cggatatctttttatctgcgcggttaac

SEQ ID NO: 15 - DNA, 46 bp, Artificial Sequence
  sPD1-Fc forward primer
agtgaattcagtgctagcagtaagcttatgtgggtccggcaggtac

SEQ ID NO: 16 - DNA, 31 bp, Artificial Sequence
  sPD1-Fc reverse primer
actttaattaatcatttacccggagtccggg

SEQ ID NO: 17 - DNA, 36 bp, Artificial Sequence
  p7.5 forward primer
gaattcatcgagctctccaaacccacccgcttttta

SEQ ID NO: 18 - DNA, 31 bp, Artificial Sequence; identical to SEQ ID NO: 16
  p7.5 reverse primer

SEQ ID NO: 19 - DNA, 34 bp, Artificial Sequence
  Infusion forward primer (sPD1-Fc)
aaatataatagaattcgatttgctagctccaaac

SEQ ID NO: 20 - DNA, 29 bp, Artificial Sequence
  Infusion reverse primer (sPD1-Fc)
tgggccctatgtcgacggatcccgagaaa

SEQ ID NO: 21 - DNA, 25 bp, Artificial Sequence
  VGF forward primer
aggttccgtaagcaaagaatataag

SEQ ID NO: 22 - DNA, 31 bp, Artificial Sequence
  VGF reverse primer
aggtaactagattttactttaatatgccgaa

SEQ ID NO: 23 - DNA, 25 bp, Artificial Sequence
  TK forward primer
ggaagggtcaaacttaataaaggat

SEQ ID NO: 24 - DNA, 22 bp, Artificial Sequence
  TK reverse primer
accgtgtcgctgtaacttacta

SEQ ID NO: 25 - DNA, 24 bp, Artificial Sequence
  K3L forward primer
gacgctgaacacgttaacgatagt

SEQ ID NO: 26 - DNA, 22 bp, Artificial Sequence
  K3L reverse primer
actgcgacgagatacaaccgga

SEQ ID NO: 27 - DNA, 29 bp, Artificial Sequence
  pHyb promoter forward primer
tgtcgacctagcacgcgtgtttaaacgtt

SEQ ID NO: 28 - DNA, 20 bp, Artificial Sequence
  pHyb promoter reverse primer
caacagtaccggattgccaa

SEQ ID NO: 29 - DNA, 39 bp, Artificial Sequence
  Exon2 forward primer
actgttgaatactagatgggagtgctaaaattcaagcac

SEQ ID NO: 30 - DNA, 46 bp, Artificial Sequence
  Exon2 reverse primer
ccgcgaattcactagagctcttgagaaaggaatttcaaaacttgat

SEQ ID NO: 31 - DNA, 38 bp, Artificial Sequence
  Exon3 forward primer
aattcctttctcaagatgaacttgtgtatacatttggc

SEQ ID NO: 32 - DNA, 40 bp, Artificial Sequence
  Exon3 reverse primer
gagcaagcaagatttcatacttcgcattatactgagggtt

SEQ ID NO: 33 - DNA, 25 bp, Artificial Sequence
  Exon4 forward primer
aaatcttgcttgctcctagacaatt

SEQ ID NO: 34 - DNA, 64 bp, Artificial Sequence
  Exon4 reverse primer
atccaacgcgttgggatccgcataaaaatgcataaaaatttatagtgtggagggtgaagcattg

SEQ ID NO: 35 - DNA, 34 bp, Artificial Sequence
  Infusion forward primer (PH20)
tgggccctatgtcgacctagcacgcgtgtttaaa

SEQ ID NO: 36 - DNA, 38 bp, Artificial Sequence
  Infusion reverse primer (PH20)
aaatataatagaattcgctagcgttgggatccgcataa

SEQ ID NO: 37 - DNA, 25 bp, Artificial Sequence
  VGF forward primer
aggttccgtaagcaaagaatataag

SEQ ID NO: 38 - DNA, 31 bp, Artificial Sequence; identical to SEQ ID NO: 22
  VGF reverse primer

SEQ ID NO: 39 - DNA, 25 bp, Artificial Sequence
  TK forward primer
ggaagggtcaaacttaataaaggat

SEQ ID NO: 40 - DNA, 22 bp, Artificial Sequence
  TK reverse primer
accgtgtcgctgtaacttacta

SEQ ID NO: 41 - DNA, 24 bp, Artificial Sequence
  K3L forward primer
gacgctgaacacgttaacgatagt

SEQ ID NO: 42 - DNA, 22 bp, Artificial Sequence
  K3L reverse primer
actgcgacgagatacaaccgga

SEQ ID NO: 43 - DNA, 38 bp, Artificial Sequence
  pI1L-B19R promoter forward primer
actgtcgactttgtatttaaaagttgtttggtgaactt

SEQ ID NO: 44 - DNA, 48 bp, Artificial Sequence
  pI1L-B19R promoter reverse primer
gtatctcgagtaggcctttatacggcactaaaatatttatataatatc

SEQ ID NO: 45 - DNA, 40 bp, Artificial Sequence
  Infusion forward primer (IL-12 P40)
taaaggcctactcgacatgtgtcctcagaagctaaccatc

SEQ ID NO: 46 - DNA, 49 bp, Artificial Sequence
  Infusion reverse primer (IL-12 P40)
cgacccaccaccgcccgagccaccgccaccggatcggaccctgcaggga

SEQ ID NO: 47 - DNA, 52 bp, Artificial Sequence
  Infusion forward primer (IL-12 P35)
ggcggtggtgggtcgggtggcggcggatctagggtcattccagtctctggac

SEQ ID NO: 48 - DNA, 64 bp, Artificial Sequence
  Infusion reverse primer (IL-12 P35)
gtgattgtatctcgagtagtcgacctataaaaacctataaaaactcaggcggagctcagatagc

SEQ ID NO: 49 - DNA, 47 bp, Artificial Sequence
  PCR forward primer (gusA)
atctgcagaagcttcaatactcgagatgttacgtcctgtagaaaccc

SEQ ID NO: 50 - DNA, 39 bp, Artificial Sequence
  PCR reverse primer (gusA)
cgttctagagttaattaatcattgtttgcctccctgctg

SEQ ID NO: 51 - DNA, 35 bp, Artificial Sequence
  Infusion forward primer (gusA)
tattgcacggggatcagctcgagatgttacgtcct

SEQ ID NO: 52 - DNA, 38 bp, Artificial Sequence
  Infusion reverse primer (gusA)
agtaatcgaattcccagaaaaattcattgtttgcctcc

SEQ ID NO: 53 - DNA, 25 bp, Artificial Sequence
  VGF forward primer
aggttccgtaagcaaagaatataag

SEQ ID NO: 54 - DNA, 31 bp, Artificial Sequence; identical to SEQ ID NO: 22
  VGF reverse primer

SEQ ID NO: 55 - DNA, 25 bp, Artificial Sequence
  TK forward primer
ggaagggtcaaacttaataaaggat

SEQ ID NO: 56 - DNA, 22 bp, Artificial Sequence
  TK reverse primer
accgtgtcgctgtaacttacta

SEQ ID NO: 57 - DNA, 22 bp, Artificial Sequence
  K3L forward primer
cgaatagccaaacggcgagaag

SEQ ID NO: 58 - DNA, 25 bp, Artificial Sequence
  K3L reverse primer
acggatacatgtggagcatctatta

SEQ ID NO: 59 - DNA, 55 bp, Artificial Sequence
  pSE/L-EGFP forward primer
cagataaaaattaattaaaaaaattgaaattttattttttttttttggaatataa

SEQ ID NO: 60 - DNA, 43 bp, Artificial Sequence
  pSE/L-EGFP reverse primer
agagctcagattaatatcgatttacttgtacagctcgtccatg

SEQ ID NO: 61 - DNA, 25 bp, Artificial Sequence
  VGF forward primer
aggttccgtaagcaaagaatataag

SEQ ID NO: 62 - DNA, 31 bp, Artificial Sequence; identical to SEQ ID NO: 22
  VGF reverse primer

SEQ ID NO: 63 - DNA, 25 bp, Artificial Sequence
  TK forward primer
ggaagggtcaaacttaataaaggat

SEQ ID NO: 64 - DNA, 22 bp, Artificial Sequence
  TK reverse primer
accgtgtcgctgtaacttacta

SEQ ID NO: 65 - DNA, 24 bp, Artificial Sequence
  K3L forward primer
gacgctgaacacgttaacgatagt

SEQ ID NO: 66 - DNA, 22 bp, Artificial Sequence
  K3L reverse primer
actgcgacgagatacaaccgga

SEQ ID NO: 67 - DNA, 25 bp, Artificial Sequence
  VGF forward primer
aggttccgtaagcaaagaatataag

SEQ ID NO: 68 - DNA, 31 bp, Artificial Sequence; identical to SEQ ID NO: 22
  VGF reverse primer

SEQ ID NO: 69 - DNA, 25 bp, Artificial Sequence
  TK forward primer
ggaagggtcaaacttaataaaggat

SEQ ID NO: 70 - DNA, 22 bp, Artificial Sequence
  TK reverse primer
accgtgtcgctgtaacttacta

SEQ ID NO: 71 - DNA, 22 bp, Artificial Sequence
  K3L forward primer
cgaatagccaaacggcgagaag

SEQ ID NO: 72 - DNA, 25 bp, Artificial Sequence
  K3L reverse primer
acggatacatgtggagcatctatta

SEQ ID NO: 73 - DNA, 33 bp, Artificial Sequence
  VGF-L forward primer (WR)
cgcagctgtgttatcgattgatagtggtgtcct

SEQ ID NO: 74 - DNA, 38 bp, Artificial Sequence
  VGF-L reverse primer (WR)
ctgcagcgctagcaccgcataatctgatagctggaata

SEQ ID NO: 75 - DNA, 42 bp, Artificial Sequence
  VGF-R forward primer (WR)
cgggatccgttaattaaactcgacgaactaaactacctatac

SEQ ID NO: 76 - DNA, 35 bp, Artificial Sequence
  VGF-R reverse primer (WR)
cgatatcggaaaatgtctgttagtaaataaccatc

SEQ ID NO: 77 - DNA, 30 bp, Artificial Sequence
  p11 promoter forward primer
cggctagctctagaagcgatgctacgctag

SEQ ID NO: 78 - DNA, 41 bp, Artificial Sequence
  p11 promoter reverse primer
caagcttcggttgcctcgaggaattcatttatagcatagaa

SEQ ID NO: 79 - DNA, 31 bp, Artificial Sequence
  LacZ forward primer
cgctcgagggatcccgtcgttttacaacgtc

SEQ ID NO: 80 - DNA, 61 bp, Artificial Sequence
  LacZ reverse primer
aagcttcttaattaaggatcccccctgcccggttattattatttttgacaccagaccaact

SEQ ID NO: 81 - DNA, 33 bp, Artificial Sequence
  TK-L forward primer (WR)
aggtcgacttgcgatcaataaatggatcacaac

SEQ ID NO: 82 - DNA, 45 bp, Artificial Sequence
  TK-L reverse primer (WR)
ttagctgcagtatgcggccgcaacaatgtctggaaagaactgtcc

SEQ ID NO: 83 - DNA, 24 bp, Artificial Sequence
  TK-R forward primer (WR)
cggaattctgtgagcgtatggcaa

SEQ ID NO: 84 - DNA, 30 bp, Artificial Sequence
  TK-R reverse primer (WR)
tcgggatcctcagtctcatgttctcaccgg

SEQ ID NO: 85 - DNA, 31 bp, Artificial Sequence; identical to SEQ ID NO: 13
  p7.5 forward primer

SEQ ID NO: 86 - DNA, 47 bp, Artificial Sequence
  p7.5 reverse primer
gaattcgcactagttccgatcgccgtgcaataaattagaatataccc

SEQ ID NO: 87 - DNA, 27 bp, Artificial Sequence
  EGFP forward primer
cgctcgagatggtgagcaagggcgagg

SEQ ID NO: 88 - DNA, 30 bp, Artificial Sequence
  EGFP reverse primer
tgagatctttacttgtacagctcgtccatg

SEQ ID NO: 89 - DNA, 28 bp, Artificial Sequence
  Gpt forward primer
cgactagtacacaagacaggcttgcgag

SEQ ID NO: 90 - DNA, 29 bp, Artificial Sequence
  Gpt reverse primer
cggaattcggcccactcataaatccagtt

SEQ ID NO: 91 - DNA, 121 bp, Artificial Sequence
  pSE/L promoter forward primer
cgagctgcagataaaaattaattaattacccgggtaccaggcctagatctgtcgactcgagcttatttatattccaaaaaaaaaaaataaaatttcaatttttaagcttcgggatccgcaa

SEQ ID NO: 92 - DNA, 121 bp, Artificial Sequence
  pSE/L promoter reverse primer
ttgcggatcccgaagcttaaaaattgaaattttattttttttttttggaatataaataagctcgagtcgacagatctaggcctggtacccgggtaattaattaatttttatctgcagctcg

SEQ ID NO: 93 - DNA, 82 bp, Artificial Sequence
  TF forward primer
atcggcggccgctttttatctgcgcggttaaccgcctttttatccatcaggtgatctgtttttattgtggagctgcagcgat

SEQ ID NO: 94 - DNA, 82 bp, Artificial Sequence
  TF reverse primer
atcgctgcagctccacaataaaaacagatcacctgatggataaaaaggcggttaaccgcgcagataaaaagcggccgccgat

SEQ ID NO: 95 - DNA, 27 bp, Artificial Sequence
  K3L-Li forward primer
tgtacgtatatttagatgttttcagct

SEQ ID NO: 96 - DNA, 27 bp, Artificial Sequence
  K3L-Li reverse primer
ataagcttcttgcattttgttattcgt

SEQ ID NO: 97 - DNA, 27 bp, Artificial Sequence
  K3L-Ri forward primer
cgcagataaaaacatatccttgttaac

SEQ ID NO: 98 - DNA, 27 bp, Artificial Sequence
  K3L-Ri reverse primer
gttaacaaggatatgtttttatctgcg

SEQ ID NO: 99 - DNA, 25 bp, Artificial Sequence
  VGF forward primer
aggttccgtaagcaaagaatataag

SEQ ID NO: 100 - DNA, 31 bp, Artificial Sequence; identical to SEQ ID NO: 22
  VGF reverse primer

SEQ ID NO: 101 - DNA, 25 bp, Artificial Sequence
  TK forward primer
ggaagggtcaaacttaataaaggat

SEQ ID NO: 102 - DNA, 22 bp, Artificial Sequence
  TK reverse primer
accgtgtcgctgtaacttacta

SEQ ID NO: 103 - DNA, 22 bp, Artificial Sequence
  K3L forward primer
cgaatagccaaacggcgagaag

SEQ ID NO: 104 - DNA, 25 bp, Artificial Sequence
  K3L reverse primer
acggatacatgtggagcatctatta

SEQ ID NO: 105 - DNA, 38 bp, Artificial Sequence
  VGF-L forward primer (Lister)
atgaagctttaaaacttgtctgtatatgtaagatgttt

SEQ ID NO: 106 - DNA, 59 bp, Artificial Sequence
  VGF-L reverse primer (Lister)
acccgggtttaattaacatgctagcgtgtaaataatataaaaataacaatacaatattg

SEQ ID NO: 107 - DNA, 57 bp, Artificial Sequence
  VGF-R forward primer (Lister)
gcttaattaaggcggccgctttttataaattttttttatgagtatttttacaaaaat

SEQ ID NO: 108 - DNA, 36 bp, Artificial Sequence
  VGF-R reverse primer (Lister)
tcccgggcatcgatagtacaataacttttatgaaat

SEQ ID NO: 109 - DNA, 72 bp, Artificial Sequence
  TK-L forward primer (Lister)
ccccgggataggatccatagtcgactttaattaatgcggccgcatgacaataaagaattaattattgttcac

SEQ ID NO: 110 - DNA, 29 bp, Artificial Sequence
  TK-L reverse primer (Lister)
agactagtccctcttcaagaacccattag

SEQ ID NO: 111 - DNA, 34 bp, Artificial Sequence
  TK-R forward primer (Lister)
ccccggggctttagtagtaggaaatgttttattg

SEQ ID NO: 112 - DNA, 55 bp, Artificial Sequence
  TK-R reverse primer (Lister)
taaggatcctctgctagctattatattttttatctaaaaaactaaaaataaacat

SEQ ID NO: 113 - DNA, 42 bp, Artificial Sequence
  K3L-L forward primer (Lister)
cactatagaactcgagcatatgtttaaacgacgcattatctg

SEQ ID NO: 114 - DNA, 42 bp, Artificial Sequence
  K3L-L reverse primer (Lister)
tgggtttggaaagctttttttataccgaacataaaaataagg

SEQ ID NO: 115 - DNA, 41 bp, Artificial Sequence
  K3L-R forward primer (Lister)
cgcagataaaaagatatccttgttaacgggctcgtaaattg

SEQ ID NO: 116 - DNA, 45 bp, Artificial Sequence
  K3L-R reverse primer (Lister)
ggagaccggcagatcttgataatacacatatttatttaggaagcg

SEQ ID NO: 117 - DNA, 25 bp, Artificial Sequence
  VGF forward primer
aggttccgtaagcaaagaatataag

SEQ ID NO: 118 - DNA, 31 bp, Artificial Sequence; identical to SEQ ID NO: 22
  VGF reverse primer

SEQ ID NO: 119 - DNA, 25 bp, Artificial Sequence
  TK forward primer
ggaagggtcaaacttaataaaggat

SEQ ID NO: 120 - DNA, 22 bp, Artificial Sequence
  TK reverse primer
accgtgtcgctgtaacttacta

SEQ ID NO: 121 - DNA, 24 bp, Artificial Sequence
  K3L forward primer
gacgctgaacacgctaacgatagt

SEQ ID NO: 122 - DNA, 22 bp, Artificial Sequence
  K3L reverse primer
actgcgacgagatacaaccgga

SEQ ID NO: 123 - protein, 5 aa, Artificial Sequence
  linker
GGGGS

SEQ ID NO: 124 - protein, 30 aa, Artificial Sequence
  linker
GGGGSGGGGSGGGGSEPKSCDKTHTCPPCP

SEQ ID NO: 125 - protein, 37 aa, Artificial Sequence
  linker
SPKAQAGGGGSAQPQAEGSLGGGGSAKASAPAGGGGS

SEQ ID NO: 126 - protein, 20 aa, Artificial Sequence
  linker
GGSGGSGGSGGSGGSEQEER

SEQ ID NO: 127 - protein, 13 aa, Artificial Sequence
  linker
GGGGSGGGGSGGS

SEQ ID NO: 128 - protein, 25 aa, Artificial Sequence
  linker
SGGGGSGGGGSGGGGSGTHTCPPCP

SEQ ID NO: 129 - protein, 8 aa, Artificial Sequence
  linker
GGSGGGGS

SEQ ID NO: 130 - protein, 14 aa, Artificial Sequence
  linker
GGGGSGGGGSGGGS

SEQ ID NO: 131 - protein, 168 aa, Artificial Sequence
  sPD-1
MWVRQVPWSFTWAVLQLSWQSGWLLEVPNGPWRSLTFYPAWLTVSEGANATFTCSLSNWSEDLMLNWNRLSPSNQTEKQAAFCNGLSQPVQDARFQIIQLPNRHDFHMNILDTRRNDSGIYLCGAISLHPKAKIEESPGAELVVTERILETSTRYPSPSPKPEGRFQG

SEQ ID NO: 132 - DNA, 504 bp, Artificial Sequence
  sPD-1
atgtgggtccggcaggtaccctggtcattcacttgggctgtgctgcagttgagctggcaatcagggtggcttctagaggtccccaatgggccctggaggtccctcaccttctacccagcctggctcacagtgtcagagggagcaaatgccaccttcacctgcagcttgtccaactggtcggaggatcttatgctgaactggaaccgcctgagtcccagcaaccagactgaaaaacaggccgccttctgtaatggtttgagccaacccgtccaggatgcccgcttccagatcatacagctgcccaacaggcatgacttccacatgaacatccttgacacacggcgcaatgacagtggcatctacctctgtggggccatctccctgcaccccaaggcaaaaatcgaggagagccctggagcagagctcgtggtaacagagagaatcctggagacctcaacaagatatcccagcccctcgcccaaaccagaaggccggtttcaagga

SEQ ID NO: 133 - protein, 405 aa, Artificial Sequence
  sPD1-Fc
MWVRQVPWSFTWAVLQLSWQSGWLLEVPNGPWRSLTFYPAWLTVSEGANATFTCSLSNWSEDLMLNWNRLSPSNQTEKQAAFCNGLSQPVQDARFQIIQLPNRHDFHMNILDTRRNDSGIYLCGAISLHPKAKIEESPGAELVVTERILETSTRYPSPSPKPEGRFQGGGGRSPRGPTIKPCPPCKCPAPNLLGGPSVFIFPPKIKDVLMISLSPIVTCVVVDVSEDDPDVQISWFVNNVEVHTAQTQTHREDYNSTLRVVSALPIQHQDWMSGKEFKCKVNNKDLPAPIERTISKPKGSVRAPQVYVLPPPEEEMTKKQVTLTCMVTDFMPEDIYVEWTNNGKTELNYKNTEPVLDSDGSYFMYSKLRVEKKNWVERNSYSCSVVHEGLHNHHTTKSFSRTPGK

SEQ ID NO: 134 - DNA, 1218 bp, Artificial Sequence
  sPD1-Fc
atgtgggtccggcaggtaccctggtcattcacttgggctgtgctgcagttgagctggcaatcagggtggcttctagaggtccccaatgggccctggaggtccctcaccttctacccagcctggctcacagtgtcagagggagcaaatgccaccttcacctgcagcttgtccaactggtcggaggatcttatgctgaactggaaccgcctgagtcccagcaaccagactgaaaaacaggccgccttctgtaatggtttgagccaacccgtccaggatgcccgcttccagatcatacagctgcccaacaggcatgacttccacatgaacatccttgacacacggcgcaatgacagtggcatctacctctgtggggccatctccctgcaccccaaggcaaaaatcgaggagagccctggagcagagctcgtggtaacagagagaatcctggagacctcaacaagatatcccagcccctcgcccaaaccagaaggccggtttcaaggaggaggaggaagatctcccagagggcccacaatcaagccctgtcctccatgcaaatgcccagcacctaacctcttgggtggaccatccgtcttcatcttccctccaaagatcaaggatgtactcatgatctccctgagccccatagtcacatgtgtggtggtggatgtgagcgaggatgacccagatgtccagatcagctggtttgtgaacaacgtggaagtacacacagctcagacacaaacccatagagaggattacaacagtactctccgggtggtcagtgccctccccatccagcaccaggactggatgagtggcaaggagttcaaatgcaaggtcaacaacaaagacctcccagcgcccatcgagagaaccatctcaaaacccaaagggtcagtaagagctccacaggtatatgtcttgcctccaccagaagaagagatgactaagaaacaggtcactctgacctgcatggtcacagacttcatgcctgaagacatttacgtggagtggaccaacaacgggaaaacagagctaaactacaagaacactgaaccagtcctggactctgatggttcttacttcatgtacagcaagctgagagtggaaaagaagaactgggtggaaagaaatagctactcctgttcagtggtccacgagggtctgcacaatcaccacacgactaagagcttctcccggactccgggtaaatga

SEQ ID NO: 135 - protein, 489 aa, Artificial Sequence
  hyaluronidase
MGVLKFKHIFFRSFVKSSGVSQIVFTFLLIPCCLTLNFRAPPVIPNVPFLWAWNAPSEFCLGKFDEPLDMSLFSFIGSPRINATGQGVTIFYVDRLGYYPYIDSITGVTVNGGIPQKISLQDHLDKAKKDITFYMPVDNLGMAVIDWEEWRPTWARNWKPKDVYKNRSIELVQQQNVQLSLTEATEKAKQEFEKAGKDFLVETIKLGKLLRPNHLWGYYLFPDCYNHHYKKPGYNGSCFNVEIKRNDDLSWLWNESTALYPSIYLNTQQSPVAATLYVRNRVREAIRVSKIPDAKSPLPVFAYTRIVFTDQVLKFLSQDELVYTFGETVALGASGIVIWGTLSIMRSMKSCLLLDNYMETILNPYIINVTLAAKMCSQVLCQEQGVCIRKNWNSSDYLHLNPDNFAIQLEKGGKFTVRGKPTLEDLEQFSEKFYCSCYSTLSCKEKADVKDTDAVDVCIADGVCIDAFLKPPMETEEPQIFYNASPSTL

SEQ ID NO: 136 - DNA, 1470 bp, Artificial Sequence
  hyaluronidase
atgggagtgctaaaattcaagcacatctttttcagaagctttgttaaatcaagtggagtatcccagatagttttcaccttccttctgattccatgttgcttgactctgaatttcagagcacctcctgttattccaaatgtgcctttcctctgggcctggaatgccccaagtgaattttgtcttggaaaatttgatgagccactagatatgagcctcttctctttcataggaagcccccgaataaacgccaccgggcaaggtgttacaatattttatgttgatagacttggctactatccttacatagattcaatcacaggagtaactgtgaatggaggaatcccccagaagatttccttacaagaccatctggacaaagctaagaaagacattacattttatatgccagtagacaatttgggaatggctgttattgactgggaagaatggagacccacttgggcaagaaactggaaacctaaagatgtttacaagaataggtctattgaattggttcagcaacaaaatgtacaacttagtctcacagaggccactgagaaagcaaaacaagaatttgaaaaggcagggaaggatttcctggtagagactataaaattgggaaaattacttcggccaaatcacttgtggggttattatctttttccggattgttacaaccatcactataagaaacccggttacaatggaagttgcttcaatgtagaaataaaaagaaatgatgatctcagctggttgtggaatgaaagcactgctctttacccatccatttatttgaacactcagcagtctcctgtagctgctacactctatgtgcgcaatcgagttcgggaagccatcagagtttccaaaatacctgatgcaaaaagtccacttccggtttttgcatatacccgcatagtttttactgatcaagttttgaaattcctttctcaagatgaacttgtgtatacatttggcgaaactgttgctctgggtgcttctggaattgtaatatggggaaccctcagtataatgcgaagtatgaaatcttgcttgctcctagacaattacatggagactatactgaatccttacataatcaacgtcacactagcagccaaaatgtgtagccaagtgctttgccaggagcaaggagtgtgtataaggaaaaactggaattcaagtgactatcttcacctcaacccagataattttgctattcaacttgagaaaggtggaaagttcacagtacgtggaaaaccgacacttgaagacctggagcaattttctgaaaaattttattgcagctgttatagcaccttgagttgtaaggagaaagctgatgtaaaagacactgatgctgttgatgtgtgtattgctgatggtgtctgtatagatgcttttctaaaacctcccatggagacagaagaacctcaaattttctacaatgcttcaccctccacactataa

SEQ ID NO: 137 - protein, 543 aa, Artificial Sequence
  IL-12
MCPQKLTISWFAIVLLVSPLMAMWELEKDVYVVEVDWTPDAPGETVNLTCDTPEEDDITWTSDQRHGVIGSGKTLTITVKEFLDAGQYTCHKGGETLSHSHLLLHKKENGIWSTEILKNFKNKTFLKCEAPNYSGRFTCSWLVQRNMDLKFNIKSSSSSPDSRAVTCGMASLSAEKVTLDQRDYEKYSVSCQEDVTCPTAEETLPIELALEARQQNKYENYSTSFFIRDIIKPDPPKNLQMKPLKNSQVEVSWEYPDSWSTPHSYFSLKFFVRIQRKKEKMKETEEGCNQKGAFLVEKTSTEVQCKGGNVCVQAQDRYYNSSCSKWACVPCRVRSGGGGSGGGGSGGGGSRVIPVSGPARCLSQSRNLLKTTDDMVKTAREKLKHYSCTAEDIDHEDITRDQTSTLKTCLPLELHKNESCLATRETSSTTRGSCLPPQKTSLMMTLCLGSIYEDLKMYQTEFQAINAALQNHNHQQIILDKGMLVAIDELMQSLNHNGETLRQKPPVGEADPYRVKMKLCILLHAFSTRVVTINRVMGYLSSA

SEQ ID NO: 138 - DNA, 45 bp, Artificial Sequence
  linker
ggtggcggtggctcgggcggtggtgggtcgggtggcggcggatct

SEQ ID NO: 139 - DNA, 582 bp, Artificial Sequence
  alpha-subunit
agggtcattccagtctctggacctgccaggtgtcttagccagtcccgaaacctgctgaagaccacagatgacatggtgaagacggccagagaaaagctgaaacattattcctgcactgctgaagacatcgatcatgaagacatcacacgggaccaaaccagcacattgaagacctgtttaccactggaactacacaagaacgagagttgcctggctactagagagacttcttccacaacaagagggagctgcctgcccccacagaagacgtctttgatgatgaccctgtgccttggtagcatctatgaggacttgaagatgtaccagacagagttccaggccatcaacgcagcacttcagaatcacaaccatcagcagatcattctagacaagggcatgctggtggccatcgatgagctgatgcagtctctgaatcataatggcgagactctgcgccagaaacctcctgtgggagaagcagacccttacagagtgaaaatgaagctctgcatcctgcttcacgccttcagcacccgcgtcgtgaccatcaacagggtgatgggctatctgagctccgcctga

SEQ ID NO: 140 - DNA, 1005 bp, Artificial Sequence
  beta-subunit
atgtgtcctcagaagctaaccatctcctggtttgccatcgttttgctggtgtctccactcatggccatgtgggagctggagaaagacgtttatgttgtagaggtggactggactcccgatgcccctggagaaacagtgaacctcacctgtgacacgcctgaagaagatgacatcacctggacctcagaccagagacatggagtcataggctctggaaagaccctgaccatcactgtcaaagagtttctagatgctggccagtacacctgccacaaaggaggcgagactctgagccactcacatctgctgctccacaagaaggaaaatggaatttggtccactgaaattttaaaaaatttcaaaaacaagactttcctgaagtgtgaagcaccaaattactccggacggttcacgtgctcatggctggtgcaaagaaacatggacttgaagttcaacatcaagagcagtagcagttcccccgactctcgggcagtgacatgtggaatggcgtctctgtctgcagagaaggtcacactggaccaaagggactatgagaagtattcagtgtcctgccaggaggatgtcacctgcccaactgccgaggagaccctgcccattgaactggcgttggaagcacggcagcagaataaatatgagaactacagcaccagcttcttcatcagggacatcatcaaaccagacccgcccaagaacttgcagatgaagcctttgaagaactcacaggtggaggtcagctgggagtaccctgactcctggagcactccccattcctacttctccctcaagttctttgttcgaatccagcgcaagaaagaaaagatgaaggagacagaggaggggtgtaaccagaaaggtgcgttcctcgtagagaagacatctaccgaagtccaatgcaaaggcgggaatgtctgcgtgcaagctcaggatcgctattacaattcctcatgcagcaagtgggcatgtgttccctgcagggtccgatcc

SEQ ID NO: 141 - protein, 140 aa, Artificial Sequence
  VGF
MSMKYLMLLFAAMIIRSFADSGNAIETTLPEITNATTDIPAIRLCGPEGDGYCLHGDCIHARDIDGMYCRCSHGYTGIRCQHVVLVDYQRSEKPNTTTSYIPSPGIVLVLVGIIIMCCLLSVYRFTRRTNKLPLQDMVVP

SEQ ID NO: 142 - DNA, 423 bp, Artificial Sequence
  VGF
atgtcgatgaaatatctgatgttgttgttcgctgctatgataatcagatcattcgccgatagtggtaacgctatcgaaacgacattgccagaaattacaaacgctacaacagatattccagctatcagattatgcggtccagagggagatggatattgtttacacggtgactgtatccacgctagagatatcgacggtatgtattgtagatgctctcatggttatacaggcattagatgtcagcatgtagtattagtagactatcaacgttcagaaaaaccaaacactacaacgtcatatatcccatctcccggtattgtgcttgtattagtaggcattattattatgtgttgtctattatctgtttataggttcactcgaagaactaataaactacctctacaagatatggttgtgccataa

SEQ ID NO: 143 - protein, 177 aa, Artificial Sequence
  TK
MNGGHIQLIIGPMFSGKSTELIRRVRRYQIAQYKCVTIKYSNDNRYGTGLWTHDKNNFEALEATKLCDVLESITDFSVIGIDEGQFFPDIVEFCERMANEGKIVIVAALDGTFQRKPFNNILNLIPLSEMVVKLTAVCMKCFKEASFSKRLGEETEIEIIGGNDMYQSVCRKCYIDS

SEQ ID NO: 144 - DNA, 534 bp, Artificial Sequence
  TK
atgaacggcggacatattcagttgataatcggccccatgttttcaggtaaaagtacagaattaattagacgagttagacgttatcaaatagctcaatataaatgcgtgactataaaatattctaacgataatagatacggaacgggactatggacgcatgataagaataattttgaagcattggaagcaactaaactatgtgatgtcttggaatcaattacagatttctccgtgataggtatcgatgaaggacagttctttccagacattgttgaattctgtgagcgtatggcaaacgaaggaaaaatagttatagtagccgcactcgatgggacatttcaacgtaaaccgtttaataatattttgaatcttattccattatctgaaatggtggtaaaactaactgctgtgtgtatgaaatgctttaaggaggcttccttttctaaacgattgggtgaggaaaccgagatagaaataataggaggtaatgatatgtatcaatcggtgtgtagaaagtgttacatcgactcataa

SEQ ID NO: 145 - protein, 88 aa, Artificial Sequence
  K3L
MLAFCYSLPNAGDVIKGRVYEKDYALYIYLFDYPHSEAILAESVKMHMDRYVEYRDKLVGKTVKVKVIRVDYTKGYIDVNYKRMCRHQ

SEQ ID NO: 146 - DNA, 267 bp, Artificial Sequence
  K3L
ttattgatgtctacacatccttttgtaattgacatctatatatccttttgtataatcaactctaatcactttaacttttacagttttccctaccagtttatccctatattcaacatatctatccatatgcatcttaacactctctgccaagatagcttcagagtgaggatagtcaaaaagataaatatatagagcataatccttctcgtatactctgccctttattacatcgcccgcattgggcaacgaataacaaaatgcaagcat